European Patent Specification EP 3 197 486 B1, published April 15, 2026. Title: FMDV RECOMBINANT VACCINES AND USES THEREOF. Applicant: Merial, Inc. AUDONNET, Jean-Christophe MEBATSION, Teshome HANNAS, Zahia CHIANG, Yu-Wei WIDENER, Justin. The sequence listing filed with the application follows.

SEQUENCE LISTING (20 sequences)

SEQ ID NO: 1 - protein, 2333 aa, artificial sequence
  Wild-type polyprotein of A24 Cruzeiro Strain (GenBank AAT01711)
MNTTDCFIALVHAIREIRAFFLPRATGRMEFTLHNGERKVFYSRPNNHDNCWLNTILQLFRYVGEPFFDWVYDSPENLTLEAIEQLEELTGLELHEGGPPALVIWNIKHLLHTGIGTASRPSEVCMVDGTNMCLADFHAGIFLKGQEHAVFACVTSNGWYAIDDEDFYPWTPDPSDVLVFVPYDQEPLNGEWKTKVQQKLKGAGQSSPATGSQNQSGNTGSIINNYYMQQYQNSMDTQLGDNAISGGSNEGSTDTTSTHTTNTQNNDWFSKLASSAFTGLFGALLADKKTEETTLLEDRILTTRNGHTTSTTQSSVGVTHGYSTEEDHVAGPNTSGLETRVVQAERFYKKYLFDWTTDKAFGHLEKLELPSDHHGVFGHLVDSYAYMRNGWDVEVSAVGNQFNGGCLLVAMVPEWKEFDTREKYQLTLFPHQFISPRTNMTAHITVPYLGVNRYDQYKKHKPWTLVVMVVSPLTVNNTSAAQIKVYANIAPTYVHVAGELPSKEGIFPVACADGYGGLVTTDPKTADPAYGKVYNPPRTNYPGRFTNLLDVAEACPTFLCFDDGKPYVTTRTDDTRLLAKFDLSLAAKHMSNTYLSGIAQYYTQYSGTINLHFMFTGSTDSKARYMVAYIPPGVETPPDTPERAAHCIHAEWDTGLNSKFTFSIPYVSAADYAYTASDTAETINVQGWVCIYQITHGKAENDTLVVSVSAGKDFELRLPIDPRQQTTATGESADPVTTTVENYGGETQIQRRHHTDIGFIMDRFVKIQSLSPTHVIDLMQTHQHGLVGALLRAATYYFSDLEIVVRHEGNLTWVPNGAPESALLNTSNPTAYNKAPFTRLALPYTAPHRVLATVYNGTSKYAVGGSGRRGDMGSLAARVVKQLPASFNYGAIKADAIHELLVRMKRAELYCPRPLLAIEVSSQDRHKQKIIAPAKQLLNFDLLKLAGDVESNPGPFFFSDVRSNFSKLVDTINQMQEDMSTKHGPDFNRLVSAFEELATGVKAIRTGLDEAKPWYKLIKLLSRLSCMAAVAARSKDPVLVAIMLADTGLEILDSTFVVKKISDSLSSLFHVPAPVFSFGAPILLAGLVKVASSFFRSTPEDLERAEKQLKARDINDIFAILKNGEWLVKLILAIRDWIKAWIASEEKFVTTTDLVPGILEKQRDLNDPSKYKEAKEWLDNARQACLKSGNVHIANLCKVVAPAPSRSRPEPVVVCLRGKSGQGKSFLANVLAQAISTHFTGRTDSVWYCPPDPDHFDGYNQQTVVVMDDLGQNPDGKDFKYFAQMVSTTGFIPPMASLEDKGKPFNSKVIIATTNLYSGFTPRTMVCPDALNRRFHFDIDVSAKDGYKINNKLDIIKALEDTHTNPVAMFQYDCALLNGMAVEMKRMQQDMFKPQPPLQNVYQLVQEVIERVELHEKVSSHPIFKQISIPSQKSVLYFLIEKGQHEAAIEFFEGMVHDSIKEELRPLIQQTSFVKRAFKRLKENFEIVALCLTLLANIVIMIRETRKRQKMVDDAVSEYIERANITTDDKTLDEAEKNPLETSGASTVGFRERPLPGQKARNDENSEPAQPAEEQPQAEGPYAGPLERQKPLKVRAKLPQQEGPYAGPMERQKPLKVKAKAPVVKEGPYEGPVKKPVALKVKAKNLIVTESGAPPTDLQKLVMGNTKPVELILDGKTVAICCATGVFGTAYLVPRHLFAEKYDKIMLDGRAMTDSDYRVFEFEIKVKGQDMLSDAALMVLHRGNRVRDITKHFRDTARMKKGTPVVGVINNADVGRLIFSGEALTYKDIVVCMDGDTMPGLFAYKAATKAGYCGGAVLAKDGADTFIVGTHSAGGNGVGYCSCVSRSMLLKMKAHVDPEPHHEGLIVDTRDVEERVHVMRKTKLAPTVAHGVFNPEFGPAALSNKDPRLNDGVVLDEVIFSKHKGDTKMSEEDKALFRRCAADYASRLHSVLGTANAPLSIYEAIKGVDGLDAMEPDTAPGLPWALQGKRRGALIDFENGTVGPEVEAALKLMEKREYKFACQTFLKDEIRPMEKVRAGKTRIVDVLPVEHILYTRMMIGRFCAQMHSNNGPQIGSAVGCNPDVDWQRFGTHFAQYRNVWDVDYSAFDANHCSDAMNIMFEEVFRTEFGFHPNAEWILKTLVNTEHAYENKRITVEGGMPSGCSATSIINTILNNIYVLYALRRHYEGVELDTYTMISYGDDIVVASDYDLDFEALKPHFKSLGQTITPADKSDKGFVLGHSITDVTFLKRHFHMDYGTGFYKPVMASKTLEAILSFARRGTIQEKLISVAGLAVHSGPDEYRRLFEPFQGLFEIPSYRSLYLRWVNAVCGDA

SEQ ID NO: 2 - protein, 1126 aa, artificial sequence
  Modified polyprotein of A24 Cruzeiro Strain in VP2 (H93C) or P1 (H179C)
MGAGQSSPATGSQNQSGNTGSIINNYYMQQYQNSMDTQLGDNAISGGSNEGSTDTTSTHTTNTQNNDWFSKLASSAFTGLFGALLADKKTEETTLLEDRILTTRNGHTTSTTQSSVGVTHGYSTEEDHVAGPNTSGLETRVVQAERFYKKYLFDWTTDKAFGHLEKLELPSDHHGVFGCLVDSYAYMRNGWDVEVSAVGNQFNGGCLLVAMVPEWKEFDTREKYQLTLFPHQFISPRTNMTAHITVPYLGVNRYDQYKKHKPWTLVVMVVSPLTVNNTSAAQIKVYANIAPTYVHVAGELPSKEGIFPVACADGYGGLVTTDPKTADPAYGKVYNPPRTNYPGRFTNLLDVAEACPTFLCFDDGKPYVTTRTDDTRLLAKFDLSLAAKHMSNTYLSGIAQYYTQYSGTINLHFMFTGSTDSKARYMVAYIPPGVETPPDTPERAAHCIHAEWDTGLNSKFTFSIPYVSAADYAYTASDTAETINVQGWVCIYQITHGKAENDTLVVSVSAGKDFELRLPIDPRQQTTATGESADPVTTTVENYGGETQIQRRHHTDIGFIMDRFVKIQSLSPTHVIDLMQAHQHGLVGALLRAATYYFSDLEIVVRHEGNLTWVPNGAPESALLNTSNPTAYNKAPFTRLALPYTAPHRVLATVYNGTSKYAVGGSGRRGDMGSLAARVVKQLPASFNYGAIKADAIHELLVRMKRAELYCPRPLLAIEVSSQDRHKQKIIAPAKQLLNFDLLKLAGDVESNPGPFFFADVRSNFSKLVDTINQMQEDMSTKHGPDFNRLVSAFEELATGVKAIRTGLDEAKPWYKLIKLLSRLSCMAAVAARSKDPVLVAIMLADTGLERQRPLKVRAKLPQQEGPYAGPLERQKPLKVKAKAPVVKEGPYEGPVKKPVALKVKAKNLIVTESGAPPTDLQKMVMGNTKPVELILDGKTVAICCATGVFGTAYLVPRHLFAEKYDKIMLDGRAMTDSDYRVFEFEIKVKGQDMLSDAALMVLHRGNRVRDITKHFRDTARMKKGTPVVGVVNNADVGRLIFSGEALTYKDIVVCMDGDTMPGLFAYKAATKAGYCGGAVLAKDGADTFIVGTHSAGGNGVGYCSCVSRSMLLRMKAHVDPEPQHE

SEQ ID NO: 3 - DNA, 3378 bp, artificial sequence
  Polynucleotide encoding modified polyprotein of A24
atgggtgctggccagtcctcccctgctaccggttcccagaaccagtccggcaacaccggttccatcatcaacaactactacatgcagcagtaccagaactccatggacacccagctgggagacaacgctatctccggtggttccaacgagggttccaccgacaccacctctacccacaccaccaacacccagaacaacgactggttctccaagctggcttcctccgctttcaccggcctgttcggtgctctgctggctgacaagaaaaccgaggaaaccaccctgctcgaggaccgtatcctgaccacccgtaacggtcacaccacttccaccacccagtcctccgtgggcgtgacccacggttactccaccgaagaggaccacgtggccggtcctaacacctccggcctggaaacccgtgtggtgcaggctgagcgcttctacaagaagtacctgttcgactggaccaccgacaaggctttcggtcacctggaaaagctggaactgccctccgaccaccacggcgtgttcggatgcctggtggactcctacgcttacatgcgtaacggctgggacgtggaggtgtccgctgtgggcaaccagttcaacggtggttgcctgctggtggctatggtgcccgagtggaaggaatttgacacccgcgagaagtaccagctgaccctgttcccccaccagttcatctccccccgtaccaacatgaccgctcacatcaccgtgccctacctgggcgtgaaccgttacgaccagtacaagaagcacaagccctggaccctggtggtcatggtggtgtcccccctgaccgtgaacaacacctccgctgctcagatcaaggtgtacgctaacatcgctcccacctacgtgcacgtcgccggagagctgccctccaaggaaggcatcttccccgtcgcttgcgctgacggttacggtggcctggtcaccaccgaccccaagaccgctgaccccgcttacggcaaggtgtacaacccccctcgcaccaactaccccggtcgtttcaccaacctgctggacgtggccgaggcttgccccaccttcctgtgcttcgacgacggcaagccctacgtgaccaccaggaccgacgacacccgtctgctggctaagttcgacctgtccctggctgctaagcacatgtccaacacctacctgtccggtatcgctcagtactacacccagtactccggcaccatcaacctgcacttcatgttcaccggctccaccgactccaaggctcgttacatggtggcttacatcccccctggtgtcgagactccccccgacactcctgagcgtgctgctcactgcatccacgctgagtgggacaccggcctgaactccaagttcaccttctccatcccttacgtgtccgctgctgactacgcgtacaccgcttccgacaccgctgagactatcaacgtgcagggctgggtctgcatctaccagatcacccacggcaaggctgagaacgacaccctggtcgtgtccgtgtccgccggcaaggacttcgagctgcgtctgcccatcgaccctcgtcagcagaccaccgctaccggcgagtctgctgacccagtgaccaccaccgtggagaactacggtggcgagactcagatccagcgtcgtcaccacaccgacatcggtttcatcatggaccgcttcgtgaagatccagtccctgtcccctacccacgtgatcgacctgatgcaggctcaccagcacggactcgtgggtgctctcctgcgtgctgctacctactacttctccgacctggaaatcgtcgtgcgtcacgagggcaacctgacctgggtgcccaacggtgctcctgagtccgctctgctgaacacctccaaccccaccgcttacaacaaggctcccttcacccgtctggctctgccttacaccgctccccaccgtgtgctggctaccgtgtacaacggcacctccaagtacgctgtgggcggttccggtcgtcgtggcgacatgggttccctggccgctcgtgtggtcaagcagctgcccgcttccttcaactacggtgctatcaaggctgacgctatccacgagctgttggtgcgtatgaagcgtgctgagctgtactgcccccgtcccctgctggctatcgaggtgtcctcccaggaccgtcacaagcagaagatcatcgctcccgctaagcagctgctgaacttcgacctgctgaagctggctggcgacgtcgagtccaaccccggtcccttcttcttcgctgacgtgcgttccaacttctctaagctggtggacactatcaaccagatgcaagaggacatgtccaccaagcacggtcccgacttcaaccgtctggtgtccgctttcgaggaactggctaccggcgtgaaggctatccgtaccggcctggacgaggctaagccctggtacaagctgatcaagctgctgtcccgtctgtcctgcatggctgctgtggctgctcgttccaaggaccccgtgctggtggccatcatgctggccgacaccggcttggagcgccagcgtcccctgaaggtccgcgctaagctgccccagcaggaaggcccttacgctggtcccctcgagcgtcagaagcctctgaaggtcaaggctaaggctcccgtggtcaaggaaggaccctacgagggacccgtgaagaagcccgtcgctctcaaggttaaggccaagaacctgatcgtgaccgagtccggtgctcctcccaccgacctgcaaaagatggtcatgggcaacaccaagcccgtggagctgatcctggacggcaagaccgtggctatctgctgcgctaccggtgttttcggcaccgcttacctggtgccccgtcacctgttcgctgagaagtacgacaagatcatgctggacggtcgtgctatgaccgactccgactaccgtgtgttcgagttcgagatcaaggtcaagggccaggacatgctgtccgacgctgctctgatggtgctgcaccgtggcaaccgtgtgcgtgacatcaccaagcacttccgtgacaccgctcgtatgaagaagggcacccccgtcgtcggtgtcgtgaacaacgctgacgtgggtcgtctgatcttctccggcgaggctctgacctacaaggacatcgtcgtgtgcatggacggcgacaccatgcccggactgttcgcttacaaggctgctaccaaggctggttactgcggtggtgctgtgctggccaaggacggtgctgacaccttcatcgtgggcacccactccgctggtggcaacggtgtcggttactgctcctgcgtgtcccgttccatgctgctgcgcatgaaggctcacgtggaccccgagccccagcacgag

SEQ ID NO: 4 - protein, 1126 aa, artificial sequence
  Unmodified Polyprotein of A24 Cruzeiro Strain
MGAGQSSPATGSQNQSGNTGSIINNYYMQQYQNSMDTQLGDNAISGGSNEGSTDTTSTHTTNTQNNDWFSKLASSAFTGLFGALLADKKTEETTLLEDRILTTRNGHTTSTTQSSVGVTHGYSTEEDHVAGPNTSGLETRVVQAERFYKKYLFDWTTDKAFGHLEKLELPSDHHGVFGHLVDSYAYMRNGWDVEVSAVGNQFNGGCLLVAMVPEWKEFDTREKYQLTLFPHQFISPRTNMTAHITVPYLGVNRYDQYKKHKPWTLVVMVVSPLTVNNTSAAQIKVYANIAPTYVHVAGELPSKEGIFPVACADGYGGLVTTDPKTADPAYGKVYNPPRTNYPGRFTNLLDVAEACPTFLCFDDGKPYVTTRTDDTRLLAKFDLSLAAKHMSNTYLSGIAQYYTQYSGTINLHFMFTGSTDSKARYMVAYIPPGVETPPDTPERAAHCIHAEWDTGLNSKFTFSIPYVSAADYAYTASDTAETINVQGWVCIYQITHGKAENDTLVVSVSAGKDFELRLPIDPRQQTTATGESADPVTTTVENYGGETQIQRRHHTDIGFIMDRFVKIQSLSPTHVIDLMQAHQHGLVGALLRAATYYFSDLEIVVRHEGNLTWVPNGAPESALLNTSNPTAYNKAPFTRLALPYTAPHRVLATVYNGTSKYAVGGSGRRGDMGSLAARVVKQLPASFNYGAIKADAIHELLVRMKRAELYCPRPLLAIEVSSQDRHKQKIIAPAKQLLNFDLLKLAGDVESNPGPFFFADVRSNFSKLVDTINQMQEDMSTKHGPDFNRLVSAFEELATGVKAIRTGLDEAKPWYKLIKLLSRLSCMAAVAARSKDPVLVAIMLADTGLERQRPLKVRAKLPQQEGPYAGPLERQKPLKVKAKAPVVKEGPYEGPVKKPVALKVKAKNLIVTESGAPPTDLQKMVMGNTKPVELILDGKTVAICCATGVFGTAYLVPRHLFAEKYDKIMLDGRAMTDSDYRVFEFEIKVKGQDMLSDAALMVLHRGNRVRDITKHFRDTARMKKGTPVVGVVNNADVGRLIFSGEALTYKDIVVCMDGDTMPGLFAYKAATKAGYCGGAVLAKDGADTFIVGTHSAGGNGVGYCSCVSRSMLLRMKAHVDPEPQHE

SEQ ID NO: 5 - protein, 736 aa, artificial sequence
  Wild-type polyprotein of FMDV O1 manisa strain (GenBank AAT01766)
GAGQSSPATGSQNQSGNTGSIINNYYMQQYQNSMDTQLGDNATSGGSNEGSTDTTSTHTTNTQNNDWFSKLASSAFSGLFGALLADKKTEETTLLEDRILTTRNGHTTSTTQSSVGVTYGYATAEDFVSGPNTSGLETRVAQAERFFKTHLFDWVTSDPFGRCHLLELPTDHKGVYGSLTDSYAYMRNGWDVEVTAVGNQFNGGCLLVAMVPELCSIQKRELYQLTLFPHQFINPRTNMTAHITVPFVGVNRYDQYKVHKPWTLVVMVVAPLTVNSEGAPQIKVYANIAPTNVHVAGEFPSKEGIFPVACSDGYGGLVTTDPKTADPAYGKVFNPPRNMLPGRFTNFLDVAEACPTFLHFEGDVPYVTTKTDSDRVLAQFDLSLAAKHMSNTFLAGLAQYYTQYSGTINLHFMFTGPTDAKARYMIAYAPPGMEPPKTPEAAAHCIHAEWDTGLNSKFTFSIPYLSAADYAYTASDTAETTNVQGWVCLFQITHGKADGDALVVLASAGKDFELRLPVDARTQTTSAGESADPVTATVENYGGETQVQRRQHTDVSFILDRFVKVTPKDQINVLDLMQTPAHTLVGALLRTATYYFADLEVAVKHEGNLTWVPNGAPEAALDNTTNPTAYHKAPLTRLALPYTAPHRVLATVYNGNSKYGDGTVANVRGDLQVLAQKAARALPTSFNYGAIKATRVTELLYRMKRAETYCPRPLLAIHPDQARHKQKIVAPVKQLL

SEQ ID NO: 6 - protein, 737 aa, artificial sequence
  Modified polyprotein of FMDV O1 manisa strain in VP2 (S93C) or P1 (S179C)
MGAGQSSPATGSQNQSGNTGSIINNYYMQQYQNSMDTQLGDNATSGGSNEGSTDTTSTHTTNTQNNDWFSKLASSAFSGLFGALLADKKTEETTLLEDRILTTRNGHTTSTTQSSVGVTYGYATAEDFVSGPNTSGLETRVAQAERFFKTHLFDWVTSDPFGRCHLLELPTDHKGVYGCLTDSYAYMRNGWDVEVTAVGNQFNGGCLLVAMVPELCSIQKRELYQLTLFPHQFINPRTNMTAHITVPFVGVNRYDQYKVHKPWTLVVMVVAPLTVNSEGAPQIKVYANIAPTNVHVAGEFPSKEGIFPVACSDGYGGLVTTDPKTADPAYGKVFNPPRNMLPGRFTNFLDVAEACPTFLHFEGDVPYVTTKTDSDRVLAQFDLSLAAKHMSNTFLAGLAQYYTQYSGTINLHFMFTGPTDAKARYMIAYAPPGMEPPKTPEAAAHCIHAEWDTGLNSKFTFSIPYLSAADYAYTASDTAETTNVQGWVCLFQITHGKADGDALVVLASAGKDFELRLPVDARTQTTSAGESADPVTATVENYGGETQVQRRQHTDVSFILDRFVKVTPKDQINVLDLMQTPAHTLVGALLRTATYYFADLEVAVKHEGNLTWVPNGAPEAALDNTTNPTAYHKAPLTRLALPYTAPHRVLATVYNGNSKYGDGTVANVRGDLQVLAQKAARALPTSFNYGAIKATRVTELLYRMKRAETYCPRPLLAIHPDQARHKQKIVAPVKQLL

SEQ ID NO: 7 - DNA, 2211 bp, artificial sequence
  Polynucleotide encoding modified polyprotein of FMDV O1 manisa strain
atgggtgctggccagtcctcccccgctaccggttcccagaaccagtccggcaacaccggttccatcatcaacaactactacatgcagcagtaccagaactccatggacacccagctgggcgacaacgctacctccggtggttccaacgagggttccaccgacaccacctctacccacaccaccaacacccagaacaacgactggttctccaagctggcttcctccgctttctccggcctgttcggtgctctgctggctgacaagaagaccgaggaaaccaccctgctcgaggaccgtatcctgaccacccgtaacggtcacaccacctccaccacccagtcctccgtgggtgtcacctacggttacgctaccgctgaggacttcgtgtccggtcccaacacctccggcctggaaacccgtgtggctcaggctgagcgcttcttcaagacccacctgttcgactgggtcacctccgaccccttcggtcgttgccacctgttggagctgcccaccgaccacaagggcgtgtacggttgcctgaccgactcctacgcttacatgcgtaacggctgggacgtggaagtgaccgctgtgggcaaccagttcaacggtggttgcctgctggtggctatggtgcccgagctgtgctccatccagaagcgcgagctgtaccagctgaccctgttcccccaccagttcatcaacccccgtaccaacatgaccgctcacatcaccgtgcccttcgtgggcgtgaaccgttacgaccagtacaaggtgcacaagccctggaccctggtcgtgatggtggtggctcccctgaccgtgaactccgagggtgctccccagatcaaggtgtacgctaacatcgctcccaccaacgtgcacgtggccggcgagttcccatccaaggaaggcatcttccccgtcgcttgctccgacggttacggtggcctggtcaccactgaccccaagaccgctgaccccgcttacggcaaggtgttcaacccccctcgtaacatgctgcccggtcgtttcaccaacttcttggacgtggccgaggcttgccccaccttcctgcacttcgagggcgacgtgccctacgtgaccaccaagactgactccgaccgtgtgctggctcagttcgacctgtccctggctgctaagcacatgtccaacactttcttggctggcctggctcagtactacacccagtactccggcaccatcaacctgcacttcatgttcaccggtcccaccgacgctaaggctcgttacatgatcgcttacgctccccctggcatggaaccccccaagaccccagaggctgctgctcactgcatccacgctgagtgggacaccggcctgaactccaagttcaccttctccatcccttacctgtccgctgctgactacgcctacaccgcttccgacaccgctgagactaccaacgtccagggctgggtctgcctgttccagatcacccacggcaaggctgacggcgacgctctggtggtgctggcttccgctggcaaggacttcgagctgcgtctgcccgtggacgctcgtacccagaccacctccgctggcgagtctgctgaccccgtgaccgctaccgtcgagaactacggtggcgagactcaggtgcagcgtcgtcagcacaccgacgtgtccttcatcctggaccgtttcgtgaaggtcacccccaaggaccagatcaacgtgctggacctgatgcagacccccgctcacaccctcgtgggcgctctgctgcgtaccgctacctactacttcgctgacctggaagtggctgtgaagcacgagggcaacctgacctgggtgcccaacggtgctcccgaggctgctctggacaacaccactaaccccaccgcttaccacaaggctcctctgacccgtctggctctgccttacactgctccccaccgcgtgctggctaccgtgtacaacggcaactctaagtacggcgacggcaccgtggctaacgtgcgtggcgatctgcaggtcctggctcagaaggctgctcgcgctctgcccacctccttcaactacggtgctatcaaggctacccgtgtgaccgagctgctgtaccgtatgaagcgtgctgagacttactgcccccgtcccctgctggctatccaccctgaccaggctcgtcacaagcaaaagatcgtggctcccgtgaagcagctgctg

SEQ ID NO: 8 - protein, 1126 aa, artificial sequence
  modified polyprotein of FMDV Iraq strain
MGAGQSSPATGSQNQSGNTGSIINNYYMQQYQNSMDTQLGDNAISGGSNEGSTDTTSTHTTNTQNNDWFSKLASSAFSGLFGALLADKKTEETTLLEDRILTTRNGHTTSTTQSSVGVTYGYSTQEDHVSGPNTSGLETRVVQAERFFKKHLFDWTPDKAFGHLEKLELPTDHKGVYGCLVDSFAYMRNGWDVEVSAVGNQFNGGCLLVAMVPEWKEFTPREKYQLTLFPHQFISPRTNMTAHIVVPYLGVNRYDQYKKHKPWTLVVMVVSPLTTNTVSAGQIKVYANIAPTHVHVAGELPSKEGIVPVACSDGYGGLVTTDPKTADPVYGMVYNPPRTNYPGRFTNLLDVAEACPTFLCFDEGKPYVVTRTDEQRLLAKFDVSLAAKHMSNTYLSGIAQYYAQYSGTINLHFMFTGSTDSKARYMVAYVPPGVETPPDTPEKAAHCIHAEWDTGLNSKFTFSIPYVSAADYAYTASDVAETTNVQGWVCIYQITHGKAEQDTLVVSVSAGKDFELRLPIDPRSQTTTTGESADPVTTTVENYGGETQVQRRQHTDVTFIMDRFVKIQNLNPTHVIDLMQTHQHGLVGALLRAATYYFSDLEIVVRHDGNLTWVPNGAPEAALSNTGNPTAYLKAPFTRLALPYTAPHRVLATVYNGTSKYSAGGTGRRGDLGPLAARVAAQLPASFNFGAIQATTIHELLVRMKRAELYCPRPLLAVEVSSQDRHKQKIIAPAKQLLNFDLLKLAGDVESNPGPFFFADVRSNFSKLVDTINQMQEDMSTKHGPDFNRLVSAFEELATGVKAIRTGLDEAKPWYKLIKLLSRLSCMAAVAARSKDPVLVAIMLADTGLERQRPLKVRAKLPQQEGPYAGPLERQKPLKVKAKAPVVKEGPYEGPVKKPVALKVKAKNLIVTESGAPPTDLQKMVMGNTKPVELILDGKTVAICCATGVFGTAYLVPRHLFAEKYDKIMLDGRAMTDSDYRVFEFEIKVKGQDMLSDAALMVLHRGNRVRDITKHFRDTARMKKGTPVVGVVNNADVGRLIFSGEALTYKDIVVCMDGDTMPGLFAYKAATKAGYCGGAVLAKDGADTFIVGTHSAGGNGVGYCSCVSRSMLLRMKAHVDPEPQHE

SEQ ID NO: 9 - DNA, 3378 bp, artificial sequence
  Polynucleotide encoding modified polyprotein of FMDV Iraq strain
atgggtgctggccagtcctcccccgctaccggttcccagaaccagtccggcaacaccggttccatcatcaacaactactacatgcagcagtaccagaactccatggacacccaactcggcgacaacgctatctccggtggttccaacgagggttccaccgacaccacctctacccacaccaccaacacccagaacaacgactggttctccaagctggcttcctccgctttctccggcctgttcggtgctctgctggctgacaagaagaccgaggaaaccaccctgctcgaggaccgtatcctgaccacccgtaacggtcacaccacctccaccacccagtcctccgtgggtgttacctacggttactccacccaagaggaccacgtgtccggtcccaacacctccggcctggaaacccgtgtggtgcaggctgagcgcttcttcaagaagcacctgttcgactggacccccgacaaggctttcggtcacctcgagaagctcgagctgcccaccgaccacaagggcgtgtacggttgcctggtggacagcttcgcttacatgcgtaacggctgggacgtcgaggtgtccgctgtgggcaaccagttcaacggtggttgcctgctggtggctatggtgcccgagtggaaagaattcacccctcgcgagaagtaccagctgaccctgttcccccaccagttcatctccccccgtaccaacatgaccgctcacatcgtggtgccctacctgggtgtcaaccgttacgaccagtacaagaagcacaagccctggaccctggtggttatggtggtgtctcccctgaccactaacaccgtgtccgctggccagatcaaggtgtacgctaacatcgctcccacccacgtgcacgtcgcgggcgagctgccttccaaagaaggcatcgtccccgtcgcttgctccgacggttacggtggcctggtcaccaccgaccccaagaccgctgaccccgtgtacggcatggtgtacaacccccctcgcaccaactaccccggtcgtttcaccaacctgctggacgtggccgaggcttgccccaccttcctgtgcttcgacgagggcaagccctacgtggtcacccgtaccgacgagcagcgtctgctggctaagttcgacgtgtccctggctgctaagcacatgtccaacacctacctgtccggtatcgctcagtactacgcccagtactccggcaccatcaacctgcacttcatgttcaccggctccaccgattccaaggctcgttacatggtggcttacgtgccccctggtgtcgagactccccccgacacccctgagaaggctgctcactgcatccacgctgagtgggacaccggcctgaactccaagttcaccttctccatcccttacgtgtccgccgctgactacgcttacaccgcttccgacgtcgccgagactaccaacgtgcagggctgggtctgcatctaccagatcacccacggcaaggctgagcaggacaccctggtcgtgtccgtgtctgctggcaaggacttcgaactccgtctgcccatcgacccccgttcccagaccaccaccaccggcgagtctgccgaccctgtgaccaccaccgtggaaaactacggtggcgagactcaggtgcagcgtcgtcagcacaccgacgtgaccttcatcatggaccgtttcgtgaagatccagaacctgaaccctacccacgtgatcgacctgatgcagactcaccagcacggcctcgtgggcgctctgctgcgtgctgctacctactacttctccgacctcgagatcgtcgtccgtcacgacggcaacctgacctgggtgcccaacggtgctcccgaggctgctctgtctaacaccggcaaccccaccgcttacctgaaggctcccttcacccgtctggctctgccctacaccgctccccaccgtgtgctggctaccgtgtacaacggcacctccaagtactccgctggtggcaccggtcgtcgtggcgacttgggtcctctggctgctcgtgtggctgctcagctgcccgcttccttcaacttcggtgctatccaggctaccaccatccacgaactcctcgtgcgtatgaagcgtgctgagctgtactgcccccgtcccctgctggctgtggaagtgtcctcccaggaccgtcacaagcagaagatcatcgctcccgctaagcagctgctgaacttcgacctgctgaagctggctggcgacgtggaatccaaccccggtcccttcttcttcgctgacgtgcgttccaacttctctaagctggtggacactatcaaccagatgcaagaggacatgtccaccaagcacggtcccgacttcaaccgtctggtgtccgctttcgaggaactggctaccggtgtcaaggctatccgtaccggcctggacgaggctaagccctggtacaagctgatcaagctgctgtcccgtctgtcctgcatggctgctgtcgctgctcgttccaaggaccccgtgctggtcgctatcatgctggccgacaccggcttggagcgtcagcgtcctctgaaagtccgcgctaagctgccccagcaagagggcccgtacgctggtcccctcgagcgtcagaagcccctgaaggttaaagccaaggctcccgtggtcaaagaaggcccatacgagggtcccgtgaagaagcccgtcgctctcaaggtcaaggccaagaacctgatcgtgaccgagtccggtgctccccccaccgacctgcaaaagatggtcatgggcaacaccaagcccgtcgagctgatcctggacggcaagaccgtggctatctgctgcgctaccggcgtgttcggtactgcttacctggtgccccgtcacctgttcgctgagaagtacgacaagatcatgctggacggtcgtgctatgaccgactccgactaccgtgtgttcgagttcgagatcaaagtcaagggccaggacatgctgtccgacgctgctctgatggtgctgcaccgtggcaaccgtgtgcgtgacatcaccaagcacttccgtgacaccgctcgtatgaagaagggcacccccgtcgtcggtgtcgtgaacaacgctgacgtgggtcgtctgatcttctccggcgaggctctgacctacaaggacatcgtcgtgtgcatggatggcgacaccatgcctggcctgttcgcttacaaggctgctaccaaggctggttactgcggtggtgctgtcctggctaaggacggtgctgacaccttcatcgtgggcacccactccgctggcggaaacggtgtcggttactgctcctgcgtgtcccgttccatgctgctgcgcatgaaggctcacgtggaccccgagccccagcacgag

SEQ ID NO: 10 - protein, 1122 aa, artificial sequence
  modified polyprotein of FMDV Asia strain
MGAGQSSPATGSQNQSGNTGSIINNYYMQQYQNSMDTQLGDNAISGGSNEGSTDTTSTHTNNTQNNDWFSRLASSAFSGLFGALLADKKTEETTLLEDRILTTRNGHTTSTTQSSVGVTYGYAVAEDAVSGPNTSGLETRVQQAERFFKKHLFDWTPNLAFGHCYYLELPTEHKGVYGCLMGSYAYMRNGWDIEVTAVGNQFNGGCLLVALVPELKELDTRQKYQLTLFPHQFINPRTNMTAHINVPYVGINRYDQYALHKPWTLVVMVVAPLTVKTGGSEQIKVYMNAAPTYVHVAGELPSKEGIVPVACADGYGNMVTTDPKTADPVYGKVFNPPRTNLPGRFTNFLDVAEACPTFLRFGEVPFVKTVNSGDRLLAKFDVSLAAGHMSNTYLAGLAQYYTQYSGTMNVHFMFTGPTDAKARYMVAYVPPGMTPPTDPEHAAHCIHSEWDTGLNSKFTFSIPYLSAADYAYTASDVAETTSVQGWVCIYQITHGKAEGDALVVSVSAGKDFEFRLPVDARQQTTTTGESADPVTTTVENYGGETQTARRLHTDVAFILDRFVKLTAPKNIQTLDLMQIPSHTLVGALLRSATYYFSDLEVALVHTGPVTWVPNGAPKDALNNQTNPTAYQKQPITRLALPYTAPHRVLATVYNGKTAYGETTSRRGDMAALAQRLSARLPTSFNYGAVKADTITELLIRMKRAETYCPRPLLALDTTQDRRKQEIIAPEKQVLNFDLLKLAGDVESNPGPFFFADVRSNFSKLVDTINQMQEDMSTKHGPDFNRLVSAFEELATGVKAIRTGLDEAKPWYKLIKLLSRLSCMAAVAARSKDPVLVAIMLADTGLERQRPLKVRAKLPQQEGPYAGPLERQKPLKVKAKAPVVKEGPYEGPVKKPVALKVKAKNLIVTESGAPPTDLQKMVMGNTKPVELILDGKTVAICCATGVFGTAYLVPRHLFAEKYDKIMLDGRAMTDSDYRVFEFEIKVKGQDMLSDAALMVLHRGNRVRDITKHFRDTARMKKGTPVVGVVNNADVGRLIFSGEALTYKDIVVCMDGDTMPGLFAYKAATKAGYCGGAVLAKDGADTFIVGTHSAGGNGVGYCSCVSRSMLLRMKAHVDPEPQHE

SEQ ID NO: 11 - DNA, 3366 bp, artificial sequence
  Polynucleotide encoding modified protein of FMDV Asia strain
atgggtgctggccagtcctcccctgctaccggttcccagaaccagtccggcaacaccggttccatcatcaacaactactacatgcagcagtaccagaactccatggacacccagctcggcgacaacgctatctccggtggttccaacgagggttccaccgacaccacctccacccacaccaacaacacccagaacaacgactggttctcccgtctggcttcctccgctttctccggcctgttcggtgctctgctggctgacaagaagaccgaggaaaccaccctgctcgaggaccgtatcctgaccacccgtaacggtcacaccacctctaccacccagtcctctgtgggtgtcacctacggttacgctgtggctgaggacgctgtgtccggtcccaacacctccggcctggaaacccgtgtgcagcaggctgagcgcttcttcaagaagcacctgttcgactggacccccaacctggctttcggtcactgctactacctcgagctgcccaccgagcacaagggcgtgtacggttgcctgatgggctcctacgcttacatgcgtaacggctgggacatcgaagtgaccgctgtgggcaaccagttcaacggtggttgcctgctggtggctctggtgcccgagctgaaagaactggacacccgtcagaagtaccagctgaccctgttcccccaccagttcatcaacccccgtaccaacatgaccgctcacatcaacgtgccctacgtgggtatcaaccgttacgaccagtacgctctgcacaagccctggaccctggtcgtgatggtggtggctcccctgaccgtcaagaccggtggctccgagcagatcaaggtgtacatgaacgctgctcccacctacgtgcacgtggccggcgagctgccctccaaagaaggcatcgtccccgtcgcttgcgctgacggttacggcaacatggtcaccaccgaccccaagaccgctgaccccgtgtacggcaaggtgttcaacccccctcgtaccaacctgcccggtcgttttaccaacttcctcgacgtggccgaggcttgccccaccttcctgcgtttcggcgaggtccccttcgtcaagactgtgaactccggcgaccgtctgctggctaagttcgacgtgtccctggctgctggtcacatgtccaacacctacctggctggcctggctcagtactacacccagtactccggcaccatgaacgtccacttcatgttcaccggtcccaccgacgctaaggctcgttacatggtggcttacgtgccccctggcatgaccccccctaccgaccctgaacacgctgctcactgcatccactccgagtgggacaccggcctgaactccaagttcaccttctccatcccttacctgtccgctgctgactacgcctacaccgcttccgatgtcgccgagactacctccgtgcagggctgggtttgcatctaccagatcacccacggcaaggctgagggcgacgctctggtggtgtccgtgtccgctggcaaggacttcgagttccgtctgcccgtggacgctcgtcagcagaccaccaccaccggcgagtccgctgacccagtgaccaccaccgtggaaaactacggtggcgagactcagaccgctcgtcgcctgcacaccgacgtggccttcatcctggaccgtttcgtgaagctgaccgctcccaagaacatccagaccctggacctgatgcagatcccctcccacaccctcgtgggcgctctgctgcgttccgctacctactacttctccgacctggaagtcgctctggtccacaccggtcccgtgacctgggtgcccaacggtgctcccaaggacgctctgaacaaccagaccaaccccaccgcttaccagaagcagcccatcacccgcctggctctgccttacaccgctccccaccgtgtcctggctactgtgtacaacggcaagaccgcttacggcgaaaccacctcccgtcgtggcgacatggctgctctggctcagcgtctgtccgctcgtctgcccacctccttcaactacggtgctgtgaaggctgacaccatcaccgagctgctgatccgtatgaagcgtgctgagacttactgcccccgtcccctgctggctctggacaccacccaggaccgtcgcaagcaagagatcatcgctcccgagaagcaggtcctgaacttcgacctgctgaagctggctggcgacgtcgagtccaaccccggtcccttcttcttcgctgacgtgcgttccaacttctccaagctggtggacaccatcaaccagatgcaagaggacatgtccaccaagcacggtcccgacttcaaccgtctggtgtccgctttcgaggaactggctaccggtgtcaaggctatccgtaccggcctggacgaggctaagccctggtacaagctgatcaagctgctgtcccgtctgtcctgcatggctgctgtcgctgctcgttccaaggaccccgtgctggtcgctatcatgctggccgacaccggcttggagcgccagcgtcctctgaaggttcgcgctaagctgcctcagcaagagggaccttacgctggtcccctcgagcgtcagaagcccctgaaggtcaaggctaaggctcccgtggtcaaagaaggcccctacgagggtcccgtgaagaagcccgtcgctctcaaggtcaaggccaagaacctgatcgtgaccgagtccggtgctccccccaccgacctgcaaaagatggtcatgggcaacaccaagcccgtcgagctgatcctggacggaaagaccgtggctatctgctgcgctaccggcgtgttcggaaccgcttacctggtgccccgtcacctgttcgctgagaagtacgacaagatcatgctggacggtcgtgctatgaccgactccgactaccgtgtgttcgagttcgagatcaaggtcaagggccaggacatgctctccgacgctgctctgatggtgctgcaccgtggcaaccgtgtgcgtgacatcaccaagcacttccgtgacaccgctcgtatgaagaagggcacccccgtcgtcggtgtcgtgaacaacgctgacgtgggtcgtctgatcttctccggcgaggctctgacctacaaggacatcgtcgtgtgcatggacggcgataccatgcctggcctgttcgcttacaaggctgctaccaaggctggttactgcggtggtgctgtgctggccaaggacggtgctgacaccttcatcgtgggcacccactccgctggtggcaacggtgtcggttactgctcctgcgtgtcccgttccatgctgctgcgtatgaaggctcacgtggaccccgagccccagcacgag

SEQ ID NO: 12 - protein, 1126 aa, artificial sequence
  Wild-type polyprotein of FMDV Iraq strain
MGAGQSSPATGSQNQSGNTGSIINNYYMQQYQNSMDTQLGDNAISGGSNEGSTDTTSTHTTNTQNNDWFSKLASSAFSGLFGALLADKKTEETTLLEDRILTTRNGHTTSTTQSSVGVTYGYSTQEDHVSGPNTSGLETRVVQAERFFKKHLFDWTPDKAFGHLEKLELPTDHKGVYGHLVDSFAYMRNGWDVEVSAVGNQFNGGCLLVAMVPEWKEFTPREKYQLTLFPHQFISPRTNMTAHIVVPYLGVNRYDQYKKHKPWTLVVMVVSPLTTNTVSAGQIKVYANIAPTHVHVAGELPSKEGIVPVACSDGYGGLVTTDPKTADPVYGMVYNPPRTNYPGRFTNLLDVAEACPTFLCFDEGKPYVVTRTDEQRLLAKFDVSLAAKHMSNTYLSGIAQYYAQYSGTINLHFMFTGSTDSKARYMVAYVPPGVETPPDTPEKAAHCIHAEWDTGLNSKFTFSIPYVSAADYAYTASDVAETTNVQGWVCIYQITHGKAEQDTLVVSVSAGKDFELRLPIDPRSQTTTTGESADPVTTTVENYGGETQVQRRQHTDVTFIMDRFVKIQNLNPTHVIDLMQTHQHGLVGALLRAATYYFSDLEIVVRHDGNLTWVPNGAPEAALSNTGNPTAYLKAPFTRLALPYTAPHRVLATVYNGTSKYSAGGTGRRGDLGPLAARVAAQLPASFNFGAIQATTIHELLVRMKRAELYCPRPLLAVEVSSQDRHKQKIIAPAKQLLNFDLLKLAGDVESNPGPFFFADVRSNFSKLVDTINQMQEDMSTKHGPDFNRLVSAFEELATGVKAIRTGLDEAKPWYKLIKLLSRLSCMAAVAARSKDPVLVAIMLADTGLERQRPLKVRAKLPQQEGPYAGPLERQKPLKVKAKAPVVKEGPYEGPVKKPVALKVKAKNLIVTESGAPPTDLQKMVMGNTKPVELILDGKTVAICCATGVFGTAYLVPRHLFAEKYDKIMLDGRAMTDSDYRVFEFEIKVKGQDMLSDAALMVLHRGNRVRDITKHFRDTARMKKGTPVVGVVNNADVGRLIFSGEALTYKDIVVCMDGDTMPGLFAYKAATKAGYCGGAVLAKDGADTFIVGTHSAGGNGVGYCSCVSRSMLLRMKAHVDPEPQHE

SEQ ID NO: 13 - protein, 1122 aa, artificial sequence
  Wild-type polyprotein of FMDV Asia strain
MGAGQSSPATGSQNQSGNTGSIINNYYMQQYQNSMDTQLGDNAISGGSNEGSTDTTSTHTNNTQNNDWFSRLASSAFSGLFGALLADKKTEETTLLEDRILTTRNGHTTSTTQSSVGVTYGYAVAEDAVSGPNTSGLETRVQQAERFFKKHLFDWTPNLAFGHCYYLELPTEHKGVYGSLMGSYAYMRNGWDIEVTAVGNQFNGGCLLVALVPELKELDTRQKYQLTLFPHQFINPRTNMTAHINVPYVGINRYDQYALHKPWTLVVMVVAPLTVKTGGSEQIKVYMNAAPTYVHVAGELPSKEGIVPVACADGYGNMVTTDPKTADPVYGKVFNPPRTNLPGRFTNFLDVAEACPTFLRFGEVPFVKTVNSGDRLLAKFDVSLAAGHMSNTYLAGLAQYYTQYSGTMNVHFMFTGPTDAKARYMVAYVPPGMTPPTDPEHAAHCIHSEWDTGLNSKFTFSIPYLSAADYAYTASDVAETTSVQGWVCIYQITHGKAEGDALVVSVSAGKDFEFRLPVDARQQTTTTGESADPVTTTVENYGGETQTARRLHTDVAFILDRFVKLTAPKNIQTLDLMQIPSHTLVGALLRSATYYFSDLEVALVHTGPVTWVPNGAPKDALNNQTNPTAYQKQPITRLALPYTAPHRVLATVYNGKTAYGETTSRRGDMAALAQRLSARLPTSFNYGAVKADTITELLIRMKRAETYCPRPLLALDTTQDRRKQEIIAPEKQVLNFDLLKLAGDVESNPGPFFFADVRSNFSKLVDTINQMQEDMSTKHGPDFNRLVSAFEELATGVKAIRTGLDEAKPWYKLIKLLSRLSCMAAVAARSKDPVLVAIMLADTGLERQRPLKVRAKLPQQEGPYAGPLERQKPLKVKAKAPVVKEGPYEGPVKKPVALKVKAKNLIVTESGAPPTDLQKMVMGNTKPVELILDGKTVAICCATGVFGTAYLVPRHLFAEKYDKIMLDGRAMTDSDYRVFEFEIKVKGQDMLSDAALMVLHRGNRVRDITKHFRDTARMKKGTPVVGVVNNADVGRLIFSGEALTYKDIVVCMDGDTMPGLFAYKAATKAGYCGGAVLAKDGADTFIVGTHSAGGNGVGYCSCVSRSMLLRMKAHVDPEPQHE

SEQ ID NO: 14 - DNA, 3378 bp, artificial sequence
  Polynucleotide encoding wild-type polyprotein of FMDV Iraq strain
atgggtgctggccagtcctcccccgctaccggttcccagaaccagtccggcaacaccggttccatcatcaacaactactacatgcagcagtaccagaactccatggacacccaactcggcgacaacgctatctccggtggttccaacgagggttccaccgacaccacctctacccacaccaccaacacccagaacaacgactggttctccaagctggcttcctccgctttctccggcctgttcggtgctctgctggctgacaagaagaccgaggaaaccaccctgctcgaggaccgtatcctgaccacccgtaacggtcacaccacctccaccacccagtcctccgtgggtgttacctacggttactccacccaagaggaccacgtgtccggtcccaacacctccggcctggaaacccgtgtggtgcaggctgagcgcttcttcaagaagcacctgttcgactggacccccgacaaggctttcggtcacctcgagaagctcgagctgcccaccgaccacaagggcgtgtacggtcacctggtggacagcttcgcttacatgcgtaacggctgggacgtcgaggtgtccgctgtgggcaaccagttcaacggtggttgcctgctggtggctatggtgcccgagtggaaagaattcacccctcgcgagaagtaccagctgaccctgttcccccaccagttcatctccccccgtaccaacatgaccgctcacatcgtggtgccctacctgggtgtcaaccgttacgaccagtacaagaagcacaagccctggaccctggtggttatggtggtgtctcccctgaccactaacaccgtgtccgctggccagatcaaggtgtacgctaacatcgctcccacccacgtgcacgtcgcgggcgagctgccttccaaagaaggcatcgtccccgtcgcttgctccgacggttacggtggcctggtcaccaccgaccccaagaccgctgaccccgtgtacggcatggtgtacaacccccctcgcaccaactaccccggtcgtttcaccaacctgctggacgtggccgaggcttgccccaccttcctgtgcttcgacgagggcaagccctacgtggtcacccgtaccgacgagcagcgtctgctggctaagttcgacgtgtccctggctgctaagcacatgtccaacacctacctgtccggtatcgctcagtactacgcccagtactccggcaccatcaacctgcacttcatgttcaccggctccaccgattccaaggctcgttacatggtggcttacgtgccccctggtgtcgagactccccccgacacccctgagaaggctgctcactgcatccacgctgagtgggacaccggcctgaactccaagttcaccttctccatcccttacgtgtccgccgctgactacgcttacaccgcttccgacgtcgccgagactaccaacgtgcagggctgggtctgcatctaccagatcacccacggcaaggctgagcaggacaccctggtcgtgtccgtgtctgctggcaaggacttcgaactccgtctgcccatcgacccccgttcccagaccaccaccaccggcgagtctgccgaccctgtgaccaccaccgtggaaaactacggtggcgagactcaggtgcagcgtcgtcagcacaccgacgtgaccttcatcatggaccgtttcgtgaagatccagaacctgaaccctacccacgtgatcgacctgatgcagactcaccagcacggcctcgtgggcgctctgctgcgtgctgctacctactacttctccgacctcgagatcgtcgtccgtcacgacggcaacctgacctgggtgcccaacggtgctcccgaggctgctctgtctaacaccggcaaccccaccgcttacctgaaggctcccttcacccgtctggctctgccctacaccgctccccaccgtgtgctggctaccgtgtacaacggcacctccaagtactccgctggtggcaccggtcgtcgtggcgacttgggtcctctggctgctcgtgtggctgctcagctgcccgcttccttcaacttcggtgctatccaggctaccaccatccacgaactcctcgtgcgtatgaagcgtgctgagctgtactgcccccgtcccctgctggctgtggaagtgtcctcccaggaccgtcacaagcagaagatcatcgctcccgctaagcagctgctgaacttcgacctgctgaagctggctggcgacgtggaatccaaccccggtcccttcttcttcgctgacgtgcgttccaacttctctaagctggtggacactatcaaccagatgcaagaggacatgtccaccaagcacggtcccgacttcaaccgtctggtgtccgctttcgaggaactggctaccggtgtcaaggctatccgtaccggcctggacgaggctaagccctggtacaagctgatcaagctgctgtcccgtctgtcctgcatggctgctgtcgctgctcgttccaaggaccccgtgctggtcgctatcatgctggccgacaccggcttggagcgtcagcgtcctctgaaagtccgcgctaagctgccccagcaagagggcccgtacgctggtcccctcgagcgtcagaagcccctgaaggttaaagccaaggctcccgtggtcaaagaaggcccatacgagggtcccgtgaagaagcccgtcgctctcaaggtcaaggccaagaacctgatcgtgaccgagtccggtgctccccccaccgacctgcaaaagatggtcatgggcaacaccaagcccgtcgagctgatcctggacggcaagaccgtggctatctgctgcgctaccggcgtgttcggtactgcttacctggtgccccgtcacctgttcgctgagaagtacgacaagatcatgctggacggtcgtgctatgaccgactccgactaccgtgtgttcgagttcgagatcaaagtcaagggccaggacatgctgtccgacgctgctctgatggtgctgcaccgtggcaaccgtgtgcgtgacatcaccaagcacttccgtgacaccgctcgtatgaagaagggcacccccgtcgtcggtgtcgtgaacaacgctgacgtgggtcgtctgatcttctccggcgaggctctgacctacaaggacatcgtcgtgtgcatggatggcgacaccatgcctggcctgttcgcttacaaggctgctaccaaggctggttactgcggtggtgctgtcctggctaaggacggtgctgacaccttcatcgtgggcacccactccgctggcggaaacggtgtcggttactgctcctgcgtgtcccgttccatgctgctgcgcatgaaggctcacgtggaccccgagccccagcacgag

SEQ ID NO: 15 - DNA, 3366 bp, artificial sequence
  Polynucleotide encoding wild-type polyprotein of FMDV Asia strain
atgggtgctggccagtcctcccctgctaccggttcccagaaccagtccggcaacaccggttccatcatcaacaactactacatgcagcagtaccagaactccatggacacccagctcggcgacaacgctatctccggtggttccaacgagggttccaccgacaccacctccacccacaccaacaacacccagaacaacgactggttctcccgtctggcttcctccgctttctccggcctgttcggtgctctgctggctgacaagaagaccgaggaaaccaccctgctcgaggaccgtatcctgaccacccgtaacggtcacaccacctctaccacccagtcctctgtgggtgtcacctacggttacgctgtggctgaggacgctgtgtccggtcccaacacctccggcctggaaacccgtgtgcagcaggctgagcgcttcttcaagaagcacctgttcgactggacccccaacctggctttcggtcactgctactacctcgagctgcccaccgagcacaagggcgtgtacggttccctgatgggctcctacgcttacatgcgtaacggctgggacatcgaagtgaccgctgtgggcaaccagttcaacggtggttgcctgctggtggctctggtgcccgagctgaaagaactggacacccgtcagaagtaccagctgaccctgttcccccaccagttcatcaacccccgtaccaacatgaccgctcacatcaacgtgccctacgtgggtatcaaccgttacgaccagtacgctctgcacaagccctggaccctggtcgtgatggtggtggctcccctgaccgtcaagaccggtggctccgagcagatcaaggtgtacatgaacgctgctcccacctacgtgcacgtggccggcgagctgccctccaaagaaggcatcgtccccgtcgcttgcgctgacggttacggcaacatggtcaccaccgaccccaagaccgctgaccccgtgtacggcaaggtgttcaacccccctcgtaccaacctgcccggtcgttttaccaacttcctcgacgtggccgaggcttgccccaccttcctgcgtttcggcgaggtccccttcgtcaagactgtgaactccggcgaccgtctgctggctaagttcgacgtgtccctggctgctggtcacatgtccaacacctacctggctggcctggctcagtactacacccagtactccggcaccatgaacgtccacttcatgttcaccggtcccaccgacgctaaggctcgttacatggtggcttacgtgccccctggcatgaccccccctaccgaccctgaacacgctgctcactgcatccactccgagtgggacaccggcctgaactccaagttcaccttctccatcccttacctgtccgctgctgactacgcctacaccgcttccgatgtcgccgagactacctccgtgcagggctgggtttgcatctaccagatcacccacggcaaggctgagggcgacgctctggtggtgtccgtgtccgctggcaaggacttcgagttccgtctgcccgtggacgctcgtcagcagaccaccaccaccggcgagtccgctgacccagtgaccaccaccgtggaaaactacggtggcgagactcagaccgctcgtcgcctgcacaccgacgtggccttcatcctggaccgtttcgtgaagctgaccgctcccaagaacatccagaccctggacctgatgcagatcccctcccacaccctcgtgggcgctctgctgcgttccgctacctactacttctccgacctggaagtcgctctggtccacaccggtcccgtgacctgggtgcccaacggtgctcccaaggacgctctgaacaaccagaccaaccccaccgcttaccagaagcagcccatcacccgcctggctctgccttacaccgctccccaccgtgtcctggctactgtgtacaacggcaagaccgcttacggcgaaaccacctcccgtcgtggcgacatggctgctctggctcagcgtctgtccgctcgtctgcccacctccttcaactacggtgctgtgaaggctgacaccatcaccgagctgctgatccgtatgaagcgtgctgagacttactgcccccgtcccctgctggctctggacaccacccaggaccgtcgcaagcaagagatcatcgctcccgagaagcaggtcctgaacttcgacctgctgaagctggctggcgacgtcgagtccaaccccggtcccttcttcttcgctgacgtgcgttccaacttctccaagctggtggacaccatcaaccagatgcaagaggacatgtccaccaagcacggtcccgacttcaaccgtctggtgtccgctttcgaggaactggctaccggtgtcaaggctatccgtaccggcctggacgaggctaagccctggtacaagctgatcaagctgctgtcccgtctgtcctgcatggctgctgtcgctgctcgttccaaggaccccgtgctggtcgctatcatgctggccgacaccggcttggagcgccagcgtcctctgaaggttcgcgctaagctgcctcagcaagagggaccttacgctggtcccctcgagcgtcagaagcccctgaaggtcaaggctaaggctcccgtggtcaaagaaggcccctacgagggtcccgtgaagaagcccgtcgctctcaaggtcaaggccaagaacctgatcgtgaccgagtccggtgctccccccaccgacctgcaaaagatggtcatgggcaacaccaagcccgtcgagctgatcctggacggaaagaccgtggctatctgctgcgctaccggcgtgttcggaaccgcttacctggtgccccgtcacctgttcgctgagaagtacgacaagatcatgctggacggtcgtgctatgaccgactccgactaccgtgtgttcgagttcgagatcaaggtcaagggccaggacatgctctccgacgctgctctgatggtgctgcaccgtggcaaccgtgtgcgtgacatcaccaagcacttccgtgacaccgctcgtatgaagaagggcacccccgtcgtcggtgtcgtgaacaacgctgacgtgggtcgtctgatcttctccggcgaggctctgacctacaaggacatcgtcgtgtgcatggacggcgataccatgcctggcctgttcgcttacaaggctgctaccaaggctggttactgcggtggtgctgtgctggccaaggacggtgctgacaccttcatcgtgggcacccactccgctggtggcaacggtgtcggttactgctcctgcgtgtcccgttccatgctgctgcgtatgaaggctcacgtggaccccgagccccagcacgag

SEQ ID NO: 16 - protein, 1184 aa, artificial sequence
  FMDV capsid protein in adenovirus
MGAGQSSPATGSQNQSGNTGSIINNYYMQQYQNSMDTQLGDNAISGGSNEGSTDTTSTHTTNTQNNDWFSKLASSAFTGLFGALLADKKTEETTLLEDRILTTRNGHTTSTTQSSVGVTHGYSTEEDHVAGPNTSGLETRVVQAERFYKKYLFDWTTDKAFGHLEKLELPSDHHGVFGCLVDSYAYMRNGWDVEVSAVGNQFNGGCLLVAMVPEWKEFDTREKYQLTLFPHQFISPRTNMTAHITVPYLGVNRYDQYKKHKPWTLVVMVVSPLTVNNTSAAQIKVYANIAPTYVHVAGELPSKEGIFPVACADGYGGLVTTDPKTADPAYGKVYNPPRTNYPGRFTNLLDVAEACPTFLCFDDGKPYVTTRTDDTRLLAKFDLSLAAKHMSNTYLSGIAQYYTQYSGTINLHFMFTGSTDSKARYMVAYIPPGVETPPDTPERAAHCIHAEWDTGLNSKFTFSIPYVSAADYAYTASDTAETINVQGWVCIYQITHGKAENDTLVVSVSAGKDFELRLPIDPRQQTTATGESADPVTTTVENYGGETQIQRRHHTDIGFIMDRFVKIQSLSPTHVIDLMQAHQHGLVGALLRAATYYFSDLEIVVRHEGNLTWVPNGAPESALLNTSNPTAYNKAPFTRLALPYTAPHRVLATVYNGTSKYAVGGSGRRGDMGSLAARVVKQLPASFNYGAIKADAIHELLVRMKRAELYCPRPLLAIEVSSQDRHKQKIIAPAKQLLNFDLLKLAGDVESNPGPFFFADVRSNFSKLVDTINQMQEDMSTKHGPDFNRLVSAFEELATGVKAIRTGLDEAKPWYKLIKLLSRLSCMAAVAARSKDPVLVAIMLADTGLEILDSTFVVKKISDSLSSLFHVPAPVFSFGAPILLAGLVKVASSFFRSTPEDLERAEKQRQRPLKVRAKLPQQEGPYAGPLERQKPLKVKAKAPVVKEGPYEGPVKKPVALKVKAKNLIVTESGAPPTDLQKMVMGNTKPVELILDGKTVAICCATGVFGTAYLVPRHLFAEKYDKIMLDGRAMTDSDYRVFEFEIKVKGQDMLSDAALMVLHRGNRVRDITKHFRDTARMKKGTPVVGVVNNADVGRLIFSGEALTYKDIVVTMDGDTMPGLFAYKAATKAGYCGGAVLAKDGADTFIVGTHSAGGNGVGYCSCVSRSMLLRMKAHVDPEPQHE

SEQ ID NO: 17 - DNA, 3552 bp, artificial sequence
  Codon-optimized polynucleotide encoding FMDV capsid precursor
atgggggctgggcagtcctctcccgccacaggctcacagaatcagtcaggcaacacagggtctattatcaacaattattatatgcagcagtaccagaactccatggacacccagctgggagataacgccatctccggcggaagcaatgaggggtccacagacaccacaagcacccacaccacaaacacacagaacaatgattggttcagcaagctggcctccagcgcttttaccggactcttcggggccctgctcgctgacaagaaaaccgaggaaaccacactgctcgaggatcgcatcctgaccacaaggaacggccacaccacatccaccacacagtcttcagtgggagtcacccacgggtacagcacagaggaagaccatgtggccggcccaaatacctctggactggaaacacgcgtggtccaggccgagcggttttacaagaaatatctgttcgactggaccacagataaggcctttggccacctggagaaactggaactcccttcagatcaccatggcgtgttcggatgtctggtcgactcctacgcctatatgcgcaacggctgggatgtggaagtctccgccgtgggaaaccagtttaatggaggatgcctgctcgtggctatggtcccagagtggaaggaattcgacaccagggagaaataccagctgacactctttcctcaccagttcatctcccccagaacaaacatgaccgcccatattaccgtgccatacctgggcgtcaatcgctacgaccagtataagaaacacaagccttggaccctggtggtcatggtggtctcacccctcacagtgaacaatacctccgccgctcagatcaaagtctacgccaacattgctcccacctatgtgcacgtcgccggggaactgccatccaaggagggcatcttccctgtggcctgtgctgacgggtacggagggctggtcaccacagaccccaagaccgccgatccagcttacggcaaagtgtataaccccccaaggaccaattaccccggaagattcacaaacctgctcgatgtggccgaggcttgcccaacctttctgtgtttcgacgatggaaagccttacgtgaccacaagaacagacgatacccgactgctcgccaagttcgacctgagcctcgccgctaaacacatgtctaacacctacctgtcagggatcgcccagtactatacccagtattccggcacaattaatctgcattttatgttcacaggatctaccgactcaaaggccagatacatggtggcttatatccctcccggagtcgaaacaccacctgacacccctgagcgagctgctcactgcatccatgccgaatgggataccgggctgaactccaagtttacattcagcattccctacgtgtctgccgctgactacgcctataccgctagcgatacagccgagaccatcaacgtgcaggggtgggtctgtatctaccagattacccacggcaaagccgaaaatgacacactggtggtctctgtgtcagccgggaaggacttcgagctgcgactccccatcgatccacgacagcagaccacagctaccggagagtccgctgaccctgtgaccacaaccgtcgaaaactacggcggagagacccagattcagcgccggcaccatacagacatcggctttattatggatcgcttcgtgaagatccagtccctgagccccacccacgtgattgacctcatgcaggctcaccagcatggactggtgggagctctgctccgagctgctacctactatttctccgatctggaaatcgtggtccggcatgagggaaacctgacctgggtgcctaatggggcccccgagtcagctctgctcaacacatccaatcccaccgcctacaacaaagctccattcaccagactggccctcccatatacagctcctcaccgagtgctggctaccgtctacaatggcacaagcaagtatgctgtgggaggctctggaaggagaggggacatgggcagcctcgctgctcgagtggtcaagcagctgccagcttctttcaactacggagccatcaaagccgatgctattcacgaactgctcgtgcgaatgaagcgcgccgagctgtattgccccaggccactgctcgccatcgaggtgtccagccaggacagacataagcagaaaatcattgccccagctaagcagctgctcaactttgacctgctcaaactggccggagatgtggaaagcaatcctgggcccttctttttcgccgacgtgaggtccaacttcagcaaactggtcgacaccatcaatcagatgcaggaggatatgtcaaccaagcacggccccgactttaaccggctggtgtccgccttcgaggaactcgctaccggcgtgaaggccatcaggacaggactggacgaggccaaaccatggtacaagctgatcaagctgctctctcgcctctcatgtatggctgctgtggctgctcggagcaaggaccccgtgctggtcgccatcatgctcgctgacaccggcctggagattctcgattctacatttgtggtcaagaaaatctctgactcactgtcttcactcttccacgtgccagcccctgtcttttccttcggagctccaattctgctcgctggactggtgaaagtcgcctccagctttttccggtccaccccagaggacctggaaagggccgagaagcagcgtcagagacctctgaaagtgagagctaagctcccacagcaggaaggaccttacgctggcccgttggagagacagaaaccgctgaaagtgaaagcaaaagccccggtcgtcaaggaaggaccttacgagggaccggtgaagaagcctgtcgctttgaaagtgaaagctaagaacttgatagtcactgagagtggtgccccaccgaccgacttgcaaaagatggtcatgggcaacacaaagcctgttgagctcatccttgacgggaagacagtagccatctgttgtgctactggagtgtttggcactgcttacctcgtgcctcgtcatcttttcgcagagaagtatgacaagatcatgctggatggcagagccatgacagacagtgactacagagtgtttgagtttgagattaaagtaaaaggacaggacatgctctcagacgctgcgctcatggtgctccaccgtgggaaccgcgtgagagatatcacgaaacactttcgtgatacagcaagaatgaagaaaggcacccccgtcgtcggtgtggtcaacaacgccgacgttgggagactgattttctctggtgaggccctcacctacaaggatattgtagtgaccatggacggagacaccatgcctggcctctttgcctacaaagccgccaccaaggcaggctactgtggaggagccgttctcgccaaggacggggccgacactttcatcgtcggcactcactccgcaggaggcaatggagttggatactgctcatgcgtttccaggtccatgcttctcagaatgaaggcacacgttgaccctgaaccacaacacgag

SEQ ID NO: 18 - DNA, 745 bp, artificial sequence
  CMV promoter
tttattaatagtaatcaattacggggtcattagttcatagcccatatatggagttccgcgttacataacttacggtaaatggcccgcctggctgaccgcccaacgacccccgcccattgacgtcaataatgacgtatgttcccatagtaacgccaatagggactttccattgacgtcaatgggtggagtatttacggtaaactgcccacttggcagtacatcaagtgtatcatatgccaagtacgccccctattgacgtcaatgacggtaaatggcccgcctggcattatgcccagtacatgaccttatgggactttcctacttggcagtacatctacgtattagtcatcgctattaccatggtgatgcggttttggcagtacatcaatgggcgtggatagcggtttgactcacggggatttccaagtctccaccccattgacgtcaatgggagtttgttttggcaccaaaatcaacgggactttccaaaatgtcgtaacaactccgccccattgacgcaaatgggcggtaggcgtgtacggtgggaggtctatataagcagagctcgtttagtgaaccgtcagatcgcctggagacgccatccacgctgttttgacctccatagaagacaccgggaccgatccagcctccgcggccgggaacggtgcattggaacgcggattccccgtgccaagagtgacgtaagtaccgcctatagagtctataggcccacccccttggcttc

SEQ ID NO: 19 - DNA, 104 bp, artificial sequence
  Synthetic enhancer
cttgaggtgtggcaggcttgagatctggccatacacttgagtgacaatgacatccactttgcctttctctccacaggtgtccactcccaggtccaactgcagcc

SEQ ID NO: 20 - DNA, 4579 bp, artificial sequence
  CMV promoter -synthetic enhancer- codon optimized FMDV capsid gene - SV40 PolyA in vAD3027
tttattaatagtaatcaattacggggtcattagttcatagcccatatatggagttccgcgttacataacttacggtaaatggcccgcctggctgaccgcccaacgacccccgcccattgacgtcaataatgacgtatgttcccatagtaacgccaatagggactttccattgacgtcaatgggtggagtatttacggtaaactgcccacttggcagtacatcaagtgtatcatatgccaagtacgccccctattgacgtcaatgacggtaaatggcccgcctggcattatgcccagtacatgaccttatgggactttcctacttggcagtacatctacgtattagtcatcgctattaccatggtgatgcggttttggcagtacatcaatgggcgtggatagcggtttgactcacggggatttccaagtctccaccccattgacgtcaatgggagtttgttttggcaccaaaatcaacgggactttccaaaatgtcgtaacaactccgccccattgacgcaaatgggcggtaggcgtgtacggtgggaggtctatataagcagagctcgtttagtgaaccgtcagatcgcctggagacgccatccacgctgttttgacctccatagaagacaccgggaccgatccagcctccgcggccgggaacggtgcattggaacgcggattccccgtgccaagagtgacgtaagtaccgcctatagagtctataggcccacccccttggcttccttgaggtgtggcaggcttgagatctggccatacacttgagtgacaatgacatccactttgcctttctctccacaggtgtccactcccaggtccaactgcagccgcggccgcatgggggctgggcagtcctctcccgccacaggctcacagaatcagtcaggcaacacagggtctattatcaacaattattatatgcagcagtaccagaactccatggacacccagctgggagataacgccatctccggcggaagcaatgaggggtccacagacaccacaagcacccacaccacaaacacacagaacaatgattggttcagcaagctggcctccagcgcttttaccggactcttcggggccctgctcgctgacaagaaaaccgaggaaaccacactgctcgaggatcgcatcctgaccacaaggaacggccacaccacatccaccacacagtcttcagtgggagtcacccacgggtacagcacagaggaagaccatgtggccggcccaaatacctctggactggaaacacgcgtggtccaggccgagcggttttacaagaaatatctgttcgactggaccacagataaggcctttggccacctggagaaactggaactcccttcagatcaccatggcgtgttcggatgtctggtcgactcctacgcctatatgcgcaacggctgggatgtggaagtctccgccgtgggaaaccagtttaatggaggatgcctgctcgtggctatggtcccagagtggaaggaattcgacaccagggagaaataccagctgacactctttcctcaccagttcatctcccccagaacaaacatgaccgcccatattaccgtgccatacctgggcgtcaatcgctacgaccagtataagaaacacaagccttggaccctggtggtcatggtggtctcacccctcacagtgaacaatacctccgccgctcagatcaaagtctacgccaacattgctcccacctatgtgcacgtcgccggggaactgccatccaaggagggcatcttccctgtggcctgtgctgacgggtacggagggctggtcaccacagaccccaagaccgccgatccagcttacggcaaagtgtataaccccccaaggaccaattaccccggaagattcacaaacctgctcgatgtggccgaggcttgcccaacctttctgtgtttcgacgatggaaagccttacgtgaccacaagaacagacgatacccgactgctcgccaagttcgacctgagcctcgccgctaaacacatgtctaacacctacctgtcagggatcgcccagtactatacccagtattccggcacaattaatctgcattttatgttcacaggatctaccgactcaaaggccagatacatggtggcttatatccctcccggagtcgaaacaccacctgacacccctgagcgagctgctcactgcatccatgccgaatgggataccgggctgaactccaagtttacattcagcattccctacgtgtctgccgctgactacgcctataccgctagcgatacagccgagaccatcaacgtgcaggggtgggtctgtatctaccagattacccacggcaaagccgaaaatgacacactggtggtctctgtgtcagccgggaaggacttcgagctgcgactccccatcgatccacgacagcagaccacagctaccggagagtccgctgaccctgtgaccacaaccgtcgaaaactacggcggagagacccagattcagcgccggcaccatacagacatcggctttattatggatcgcttcgtgaagatccagtccctgagccccacccacgtgattgacctcatgcaggctcaccagcatggactggtgggagctctgctccgagctgctacctactatttctccgatctggaaatcgtggtccggcatgagggaaacctgacctgggtgcctaatggggcccccgagtcagctctgctcaacacatccaatcccaccgcctacaacaaagctccattcaccagactggccctcccatatacagctcctcaccgagtgctggctaccgtctacaatggcacaagcaagtatgctgtgggaggctctggaaggagaggggacatgggcagcctcgctgctcgagtggtcaagcagctgccagcttctttcaactacggagccatcaaagccgatgctattcacgaactgctcgtgcgaatgaagcgcgccgagctgtattgccccaggccactgctcgccatcgaggtgtccagccaggacagacataagcagaaaatcattgccccagctaagcagctgctcaactttgacctgctcaaactggccggagatgtggaaagcaatcctgggcccttctttttcgccgacgtgaggtccaacttcagcaaactggtcgacaccatcaatcagatgcaggaggatatgtcaaccaagcacggccccgactttaaccggctggtgtccgccttcgaggaactcgctaccggcgtgaaggccatcaggacaggactggacgaggccaaaccatggtacaagctgatcaagctgctctctcgcctctcatgtatggctgctgtggctgctcggagcaaggaccccgtgctggtcgccatcatgctcgctgacaccggcctggagattctcgattctacatttgtggtcaagaaaatctctgactcactgtcttcactcttccacgtgccagcccctgtcttttccttcggagctccaattctgctcgctggactggtgaaagtcgcctccagctttttccggtccaccccagaggacctggaaagggccgagaagcagcgtcagagacctctgaaagtgagagctaagctcccacagcaggaaggaccttacgctggcccgttggagagacagaaaccgctgaaagtgaaagcaaaagccccggtcgtcaaggaaggaccttacgagggaccggtgaagaagcctgtcgctttgaaagtgaaagctaagaacttgatagtcactgagagtggtgccccaccgaccgacttgcaaaagatggtcatgggcaacacaaagcctgttgagctcatccttgacgggaagacagtagccatctgttgtgctactggagtgtttggcactgcttacctcgtgcctcgtcatcttttcgcagagaagtatgacaagatcatgctggatggcagagccatgacagacagtgactacagagtgtttgagtttgagattaaagtaaaaggacaggacatgctctcagacgctgcgctcatggtgctccaccgtgggaaccgcgtgagagatatcacgaaacactttcgtgatacagcaagaatgaagaaaggcacccccgtcgtcggtgtggtcaacaacgccgacgttgggagactgattttctctggtgaggccctcacctacaaggatattgtagtgaccatggacggagacaccatgcctggcctctttgcctacaaagccgccaccaaggcaggctactgtggaggagccgttctcgccaaggacggggccgacactttcatcgtcggcactcactccgcaggaggcaatggagttggatactgctcatgcgtttccaggtccatgcttctcagaatgaaggcacacgttgaccctgaaccacaacacgagtagtaggcggccgctctagactagctagaaagatccgggaacttgtttattgcagcttataatggttacaaataaagcaatagcatcacaaatttcacaaataaagcatttttttcactgcattctagttgtggtttgtccaaactcatcaatgtatcttatcatgtctg